European Patent Specification EP 3 487 882 B1, published July 16, 2025. Title: ANTI- GPRC5D ANTIBODIES, BISPECIFIC ANTIGEN BINDING MOLECULES THAT BIND GPRC5D AND CD3, AND USES THEREOF. Applicant: JANSSEN PHARMACEUTICA NV. The sequence listing filed with the application follows.

SEQUENCE LISTING (100 sequences)

SEQ ID NO: 1 - protein, 5 aa, Homo sapiens
SYAIS

SEQ ID NO: 2 - protein, 5 aa, Homo sapiens
NYWMS

SEQ ID NO: 3 - protein, 5 aa, Homo sapiens
SYFIG

SEQ ID NO: 4 - protein, 5 aa, Homo sapiens
GYTMN

SEQ ID NO: 5 - protein, 17 aa, Homo sapiens
GIIPIFGTANYAQKFQG

SEQ ID NO: 6 - protein, 17 aa, Homo sapiens
GISYSGGSKYYASSVKG

SEQ ID NO: 7 - protein, 17 aa, Homo sapiens
IIYPGKSDTRYSPSFQG

SEQ ID NO: 8 - protein, 17 aa, Homo sapiens
LINPYNSDTNYAQKLQG

SEQ ID NO: 9 - protein, 10 aa, Homo sapiens
ESRWRGYKLD

SEQ ID NO: 10 - protein, 13 aa, Homo sapiens
AAFDFGRRAVRLD

SEQ ID NO: 11 - protein, 14 aa, Homo sapiens
VYSFGGRHKALFDY

SEQ ID NO: 12 - protein, 9 aa, Homo sapiens
VALRVALDY

SEQ ID NO: 13 - protein, 11 aa, Homo sapiens
RASQSISSYLN

SEQ ID NO: 14 - protein, 11 aa, Homo sapiens
RASQSVSSYLA

SEQ ID NO: 15 - protein, 11 aa, Homo sapiens
KASQNVATHVG

SEQ ID NO: 16 - protein, 7 aa, Homo sapiens
AASSLQS

SEQ ID NO: 17 - protein, 7 aa, Homo sapiens
DASNRAT

SEQ ID NO: 18 - protein, 7 aa, Homo sapiens
SASYRYS

SEQ ID NO: 19 - protein, 9 aa, Homo sapiens
QQSYSTPLT

SEQ ID NO: 20 - protein, 9 aa, Homo sapiens
QQRSNWPLT

SEQ ID NO: 21 - protein, 9 aa, Homo sapiens
QQYNRYPYT

SEQ ID NO: 22 - protein, 345 aa, Homo sapiens
MYKDCIESTGDYFLLCDAEGPWGIILESLAILGIVVTILLLLAFLFLMRKIQDCSQWNVLPTQLLFLLSVLGLFGLAFAFIIELNQQTAPVRYFLFGVLFALCFSCLLAHASNLVKLVRGCVSFSWTTILCIAIGCSLLQIIIATEYVTLIMTRGMMFVNMTPCQLNVDFVVLLVYVLFLMALTFFVSKATFCGPCENWKQHGRLIFITVLFSIIIWVVWISMLLRGNPQFQRQPQWDDPVVCIALVTNAWVFLLLYIVPELCILYRSCRQECPLQGNACPVTAYQHSFQVENQELSRARDSDGAEEDVALTSYGTPIQPQTVDPTQECFIPQAKLSPQQDAGGV

SEQ ID NO: 23 - protein, 344 aa, Macaca fascicularis
MYKDCIESTGDYFLPCDSEGPWGIVLESLAILGIVVTILLLLAFLFLMRKIQDCSQWNVLPTQLLFLLSVLGLFGLAFAFIIQLNQQTAPVRYFLFGVLFALCFSCLLAHASNLVKLVRGRVSFSWTTILCIAIGCSLLQVIIAIEYVTLIMTRGMMFVHMTPYQLNVDFVVLLVYVLFLMALTFFVSKATFCGPCENWKQHGRLIFITVLFSIIIWVVWISMLLRGNPQFQRQPQWDDPVVCIALVTNAWVFLLLYIVPELCILYRSCRQECPSQGHACPVTAYQRSFQVENQELSRARDSDGAEEDVALTSFGTPIQPQTVDPTQECFIPRAKLSPQQDAGV

SEQ ID NO: 24 - protein, 344 aa, Mus sp.
MYEDCVKSTEDYYLFCDNEGPWAIVLESLAVIGIVVTILLLLAFLFLMRKVQDCSQWNVLPTQFLFLLAVLGLFGLTFAFIIQLNHQTAPVRYFLFGVLFAICFSCLLAHASNLVKLVRGRVSFCWTTILFIAIGVSLLQTIIAIEYVTLIMTRGLMFEHMTPYQLNVDFVCLLIYVLFLMALTFFVSKATFCGPCENWKQHGRLIFATVLVSIIIWVVWISMLLRGNPQLQRQPHWDDAVICIGLVTNAWVFLLIYIIPELSILYRSCRQECPTQGNVCQVPVYQRSFRMDTQEPTRARDSDGAQEDVALTAYGTPIQLQSADPSREYLIPSATLSPQQDAGL

SEQ ID NO: 25 - protein, 125 aa, Homo sapiens
EVQLVESGGGLVQPGGSLRLSCAASGFTFNTYAMNWVRQAPGKGLEWVARIRSKYNNYATYYAASVKGRFTISRDDSKNSLYLQMNSLKTEDTAVYYCARHGNFGNSYVSWFAYWGQGTLVTVSS

SEQ ID NO: 26 - protein, 109 aa, Homo sapiens
QTVVTQEPSLTVSPGGTVTLTCRSSTGAVTTSNYANWVQQKPGQAPRGLIGGTNKRAPGTPARFSGSLLGGKAALTLSGVQPEDEAEYYCALWYSNLWVFGGGTKLTVL

SEQ ID NO: 27 - protein, 5 aa, Homo sapiens
SYWIG

SEQ ID NO: 28 - protein, 17 aa, Homo sapiens
GISYSGGSKYYADSVKG

SEQ ID NO: 29 - protein, 17 aa, Homo sapiens
IIYPGDSDTRYSPSFQG

SEQ ID NO: 30 - protein, 14 aa, Homo sapiens
AAWDFGRRAVRLDY

SEQ ID NO: 31 - protein, 11 aa, Homo sapiens
ESRYRGYKLDY

SEQ ID NO: 32 - protein, 11 aa, Homo sapiens
ESRVRGYKLDY

SEQ ID NO: 33 - protein, 11 aa, Homo sapiens
ESRGRGYKLDY

SEQ ID NO: 34 - protein, 11 aa, Homo sapiens
ESRARGYKLDY

SEQ ID NO: 35 - protein, 11 aa, Homo sapiens
ESRFRGYKLDY

SEQ ID NO: 36 - protein, 5 aa, Homo sapiens
SYYIG

SEQ ID NO: 37 - protein, 5 aa, Homo sapiens
SYVIG

SEQ ID NO: 38 - protein, 5 aa, Homo sapiens
SYGIG

SEQ ID NO: 39 - protein, 5 aa, Homo sapiens
SYAIG

SEQ ID NO: 40 - protein, 17 aa, Homo sapiens
IIYPGASDTRYSPSFQG

SEQ ID NO: 41 - protein, 17 aa, Homo sapiens
IIYPGSSDTRYSPSFQG

SEQ ID NO: 42 - protein, 17 aa, Homo sapiens
IIYPGESDTRYSPSFQG

SEQ ID NO: 43 - protein, 17 aa, Homo sapiens
IIYPGYSDTRYSPSFQG

SEQ ID NO: 44 - protein, 17 aa, Homo sapiens
GISYSGGSKYYAASVKG

SEQ ID NO: 45 - protein, 17 aa, Homo sapiens
GISYSGGSKYYAKSVKG

SEQ ID NO: 46 - protein, 17 aa, Homo sapiens
GISYSGGSKYYAESVKG

SEQ ID NO: 47 - protein, 17 aa, Homo sapiens
GISYSGGSKYYAYSVKG

SEQ ID NO: 48 - protein, 14 aa, Homo sapiens
AAYDFGRRAVRLDY

SEQ ID NO: 49 - protein, 14 aa, Homo sapiens
AAVDFGRRAVRLDY

SEQ ID NO: 50 - protein, 14 aa, Homo sapiens
AAGDFGRRAVRLDY

SEQ ID NO: 51 - protein, 14 aa, Homo sapiens
AAADFGRRAVRLDY

SEQ ID NO: 52 - protein, 120 aa, Homo sapiens
QVQLVQSGAEVKKPGSSVKVSCKASGGTFSSYAISWVRQAPGQGLEWMGGIIPIFGTANYAQKFQGRVTITADESTSTAYMELSSLRSEDTAVYYCARESRWRGYKLDYWGQGTLVTVSS

SEQ ID NO: 53 - protein, 123 aa, Homo sapiens
EVQLLESGGGLVQPGGSLRLSCAASGFTFSNYWMSWVRQAPGKGLEWVSGISYSGGSKYYASSVKGRFTISRDNSKNTLYLQMNSLRAEDTAVYYCAKAAFDFGRRAVRLDYWGQGTLVTVSS

SEQ ID NO: 54 - protein, 123 aa, Homo sapiens
EVQLVQSGAEVKKPGESLKISCKGSGYSFTSYFIGWVRQMPGKGLEWMGIIYPGKSDTRYSPSFQGQVTISADKSISTAYLQWSSLKASDTAMYYCARVYSFGGRHKALFDYWGQGTLVTVSS

SEQ ID NO: 55 - protein, 118 aa, Homo sapiens
QVQLVQSGAEVKKPGASVKVSCKASGYSFTGYTMNWVRQAPGQGLEWMGLINPYNSDTNYAQKLQGRVTMTTDTSTSTAYMELRSLRSDDTAVYYCARVALRVALDYWGQGTLVTVSS

SEQ ID NO: 56 - protein, 107 aa, Homo sapiens [sequence omitted]

SEQ ID NO: 57 - protein, 107 aa, Homo sapiens
EIVLTQSPATLSLSPGERATLSCRASQSVSSYLAWYQQKPGQAPRLLIYDASNRATGIPARFSGSGSGTDFTLTISSLEPEDFAVYYCQQRSNWPLTFGQGTKVEIK

SEQ ID NO: 58 - protein, 107 aa, Homo sapiens
DIQMTQSPSSLSASVGDRVTITCKASQNVATHVGWYQQKPGKAPKRLIYSASYRYSGVPSRFSGSGSGTEFTLTISNLQPEDFATYYCQQYNRYPYTFGQGTKLEIK

SEQ ID NO: 59 - protein, 327 aa, Homo sapiens
ASTKGPSVFPLAPCSRSTSESTAALGCLVKDYFPEPVTVSWNSGALTSGVHTFPAVLQSSGLYSLSSVVTVPSSSLGTKTYTCNVDHKPSNTKVDKRVESKYGPPCPPCPAPEAAGGPSVFLFPPKPKDTLMISRTPEVTCVVVDVSQEDPEVQFNWYVDGVEVHNAKTKPREEQFNSTYRVVSVLTVLHQDWLNGKEYKCKVSNKGLPSSIEKTISKAKGQPREPQVYTLPPSQEEMTKNQVSLTCLVKGFYPSDIAVEWESNGQPENNYKTTPPVLDSDGSFFLYSRLTVDKSRWQEGNVFSCSVMHEALHNHYTQKSLSLSLGK

SEQ ID NO: 60 - protein, 330 aa, Homo sapiens
ASTKGPSVFPLAPSSKSTSGGTAALGCLVKDYFPEPVTVSWNSGALTSGVHTFPAVLQSSGLYSLSSVVTVPSSSLGTQTYICNVNHKPSNTKVDKKVEPKSCDKTHTCPPCPAPELLGGPSVFLFPPKPKDTLMISRTPEVTCVVVDVSHEDPEVKFNWYVDGVEVHNAKTKPREEQYNSTYRVVSVLTVLHQDWLNGKEYKCKVSNKALPAPIEKTISKAKGQPREPQVYTLPPSREEMTKNQVSLTCLVKGFYPSDIAVEWESNGQPENNYKTTPPVLDSDGSFFLYSKLTVDKSRWQQGNVFSCSVMHEALHNHYTQKSLSLSPGK

SEQ ID NO: 61 - protein, 5 aa, Homo sapiens
DYGMH

SEQ ID NO: 62 - protein, 5 aa, Homo sapiens
GYAMS

SEQ ID NO: 63 - protein, 5 aa, Homo sapiens
SYGIS

SEQ ID NO: 64 - protein, 10 aa, Homo sapiens
GYSFTGYTMN

SEQ ID NO: 65 - protein, 5 aa, Homo sapiens
SYAMS

SEQ ID NO: 66 - protein, 10 aa, Homo sapiens
GFSLTSYNVH

SEQ ID NO: 67 - protein, 17 aa, Homo sapiens
AIKYSGGSTYYADSVKG

SEQ ID NO: 68 - protein, 17 aa, Homo sapiens
AISGSGGSTYYADSVKG

SEQ ID NO: 69 - protein, 17 aa, Homo sapiens
GIIPIFGNINYAQKFQG

SEQ ID NO: 70 - protein, 10 aa, Homo sapiens
LINPYNGDTN

SEQ ID NO: 71 - protein, 16 aa, Homo sapiens
VIWAGGSTNYNSALMS

SEQ ID NO: 72 - protein, 10 aa, Homo sapiens
RAESGPGLDY

SEQ ID NO: 73 - protein, 13 aa, Homo sapiens
IGFYGRSFRIFDY

SEQ ID NO: 74 - protein, 14 aa, Homo sapiens
VDRSFGRSRYTLDY

SEQ ID NO: 75 - protein, 14 aa, Homo sapiens
VSRRFKRFAYYFDY

SEQ ID NO: 76 - protein, 10 aa, Homo sapiens
SNFLPVVFDY

SEQ ID NO: 77 - protein, 9 aa, Homo sapiens
DGIRLRFAY

SEQ ID NO: 78 - protein, 7 aa, Homo sapiens
WASTRES

SEQ ID NO: 79 - protein, 7 aa, Homo sapiens
TASNRAT

SEQ ID NO: 80 - protein, 9 aa, Homo sapiens
QQYYSTPLT

SEQ ID NO: 81 - protein, 9 aa, Homo sapiens
QQYFRAPIT

SEQ ID NO: 82 - protein, 119 aa, Homo sapiens
EVQLLESGGGLVQPGGSLRLSCAASGFTFSDYGMHWVRQAPGKGLEWVSAIKYSGGSTYYADSVKGRFTISRDNSKNTLYLQMNSLRAEDTAVYYCAKRAESGPGLDYWGQGTLVTVSS

SEQ ID NO: 83 - protein, 123 aa, Homo sapiens
EVQLLESGGGLVQPGGSLRLSCAASGFTFSNYWMSWVRQAPGKGLEWVSGISYSGGSKYYADSVKGRFTISRDNSKNTLYLQMNSLRAEDTAVYYCAKAAWDFGRRAVRLDYWGQGTLVTVSS

SEQ ID NO: 84 - protein, 122 aa, Homo sapiens
EVQLVQSGAEVKKPGESLKISCKGSGYSFTSYWIGWVRQMPGKGLEWMGIIYPGDSDTRYSPSFQGQVTISADKSISTAYLQWSSLKASDTAMYYCARIGFYGRSFRIFDYWGQGTLVTVSS

SEQ ID NO: 85 - protein, 123 aa, Homo sapiens
EVQLVQSGAEVKKPGESLKISCKGSGYSFTSYWIGWVRQMPGKGLEWMGIIYPGDSDTRYSPSFQGQVTISADKSISTAYLQWSSLKASDTAMYYCARVYSFGGRHKALFDYWGQGTLVTVSS

SEQ ID NO: 86 - protein, 123 aa, Homo sapiens
EVQLLESGGGLVQPGGSLRLSCAASGFTFSGYAMSWVRQAPGKGLEWVSAISGSGGSTYYADSVKGRFTISRDNSKNTLYLQMNSLRAEDTAVYYCAKVDRSFGRSRYTLDYWGQGTLVTVSS

SEQ ID NO: 87 - protein, 123 aa, Homo sapiens
QVQLVQSGAEVKKPGSSVKVSCKASGGTFSSYGISWVRQAPGQGLEWMGGIIPIFGNINYAQKFQGRVTITADESTSTAYMELSSLRSEDTAVYYCARVSRRFKRFAYYFDYWGQGTLVTVSS

SEQ ID NO: 88 - protein, 118 aa, Homo sapiens
QVQLVQSGAEVKKPGASVKVSCKASGYSFTGYTMNWVRQAPGQGLEWMGLINPYNGDTNYAQKLQGRVTMTTDTSTSTAYMELRSLRSDDTAVYYCARVALRVALDYWGQGTLVTVSS

SEQ ID NO: 89 - protein, 119 aa, Homo sapiens
EVQLLESGGGLVQPGGSLRLSCAASGFTFSSYAMSWVRQAPGKGLEWVSAISGSGGSTYYADSVKGRFTISRDNSKNTLYLQMNSLRAEDTAVYYCAKSNFLPVVFDYWGQGTLVTVSS

SEQ ID NO: 90 - DNA, 705 bp, Homo sapiens
atgcgggtgctggcccagctgctgggactgctgctgctgtgcttccctggcgccagatgcgacatccagatgacccagagccccagcagcctgagcgccagcgtgggcgaccgggtgaccatcacctgcaaggccagccagaacgtggccacccacgtgggctggtaccagcagaagcccggcaaggcccccaagcggctgatctacagcgccagctaccggtacagcggcgtgcccagccggttcagcggcagcggcagcggcaccgagttcaccctgaccatcagcaacctgcagcccgaggacttcgccacctactactgccagcagtacaaccggtacccctacaccttcggccagggcaccaagctggagatcaagcgtacggtggctgcaccatctgtcttcatcttcccgccatctgatgagcagttgaaatctggaactgcctctgttgtgtgcctgctgaataacttctatcccagagaggccaaagtacagtggaaggtggataacgccctccaatcgggtaactcccaggagagtgtcacagagcaggacagcaaggacagcacctacagcctcagcagcaccctgacgctgagcaaagcagactacgagaaacacaaagtctacgcctgcgaagtcacccatcagggcctgagctcgcccgtcacaaagagcttcaacaggggagagtgttga

SEQ ID NO: 91 - protein, 117 aa, Homo sapiens
QVTLKESGPVLVKPTETLTLTCTVSGFSLTSYNVHWIRQPPGKALEWLAVIWAGGSTNYNSALMSRLTISKDTSKSQVVLTMTNMRAEDTATYYCARDGIRLRFAYWGQGTLVTVSS

SEQ ID NO: 92 - protein, 113 aa, Homo sapiens
DIVMTQSPDSLAVSLGERATINCKSSQSVLYSSNNKNYLAWYQQKPGQPPKLLIYWASTRESGVPDRFSGSGSGTDFTLTISSLQAEDVAVYYCQQYYSTPLTFGQGTKVEIK

SEQ ID NO: 93 - protein, 108 aa, Homo sapiens
EIVLTQSPATLSLSPGERATLSCRASQSVRKSLAWYQQKPGQAPRLLIYTASNRATGIPARFSGSGSGTDFTLTISSLEPEDFAVYYCQQYFRAPITFGQGTKVEIKK

SEQ ID NO: 94 - protein, 107 aa, Homo sapiens
EIVMTQSPATLSVSPGERATLSCKASQNVATHVGWYQQKPGQAPRLLIYSASYRYSGIPARFSGSGSGTEFTLTISSLQSEDFAVYYCQQYNRYPYTFGQGTKLEIK

SEQ ID NO: 95 - protein, 11 aa, Homo sapiens
RASQSVRKSLA

SEQ ID NO: 96 - DNA, 1395 bp, Homo sapiens
atggcctgggtctggaccctgctgttcctgatggccgctgcccagagcatccaggcccaggtgcagctggtgcagagcggcgccgaggtgaagaagcccggcgccagcgtgaaggtgagctgcaaggccagcggctacagcttcaccggctacaccatgaactgggtgcggcaggcccccggccagggcctggagtggatgggcctgatcaacccctacaacagcgacaccaactacgcccagaagctgcagggccgggtgaccatgaccaccgacaccagcaccagcaccgcctacatggagctgcggagcctgcggagcgacgacaccgccgtgtactactgcgcccgggtggccctgcgggtggccctggactactggggccagggcaccctggtgaccgtgagcagcgcctccaccaagggcccatccgtcttccccctggcgccctgctccaggagcacctccgagagcacagccgccctgggctgcctggtcaaggactacttccccgaaccggtgacggtgtcgtggaactcaggcgccctgaccagcggcgtgcacaccttcccggctgtcctacagtcctcaggactctactccctcagcagcgtggtgaccgtgccctccagcagcttgggcacgaaaacctacacctgcaacgtagatcacaagcccagcaacaccaaggtggacaagagagttgagtccaaatatggtcccccatgcccaccatgcccagcacctgaggccgccgggggaccatcagtcttcctgttccccccaaaacccaaggacactctcatgatctcccggacccctgaggtcacgtgcgtggtggtggacgtgagccaggaagaccccgaggtccagttcaactggtacgtggatggcgtggaggtgcataatgccaagacaaagccgcgggaggagcagttcaacagcacgtaccgtgtggtcagcgtcctcaccgtcctgcaccaggactggctgaacggcaaggagtacaagtgcaaggtctccaacaaaggcctcccgtcctccatcgagaaaaccatctccaaagccaaagggcagccccgagagccacaggtgtacaccctgcccccatcccaggaggagatgaccaagaaccaggtcagcctgacctgcctggtcaaaggcttctaccccagcgacatcgccgtggagtgggagagcaatgggcagccggagaacaactacaagaccacgcctcccgtgctggactccgacggctccttcttcctctacagcaggctaaccgtggacaagagcaggtggcaggaggggaatgtcttctcatgctccgtgatgcatgaggctctgcacaaccactacacacagaagagcctctccctgtctctgggtaaatga

SEQ ID NO: 97 - protein, 14 aa, Homo sapiens
AAFDFGRRAVRLDY

SEQ ID NO: 98 - protein, 17 aa, Homo sapiens
KSSQSVLYSSNNKNYLA

SEQ ID NO: 99 - protein, 452 aa, Artificial Sequence
  source: /note="Description of Artificial Sequence: Synthetic polypeptide"
EVQLVESGGGLVQPGGSLRLSCAASGFTFNTYAMNWVRQAPGKGLEWVARIRSKYNNYATYYAASVKGRFTISRDDSKNSLYLQMNSLKTEDTAVYYCARHGNFGNSYVSWFAYWGQGTLVTVSSASTKGPSVFPLAPCSRSTSESTAALGCLVKDYFPEPVTVSWNSGALTSGVHTFPAVLQSSGLYSLSSVVTVPSSSLGTKTYTCNVDHKPSNTKVDKRVESKYGPPCPPCPAPEAAGGPSVFLFPPKPKDTLMISRTPEVTCVVVDVSQEDPEVQFNWYVDGVEVHNAKTKPREEQFNSTYRVVSVLTVLHQDWLNGKEYKCKVSNKGLPSSIEKTISKAKGQPREPQVYTLPPSQEEMTKNQVSLTCLVKGFYPSDIAVEWESNGQPENNYKTTPPVLDSDGSFLLYSKLTVDKSRWQEGNVFSCSVMHEALHNHYTQKSLSLSLGK

SEQ ID NO: 100 - protein, 215 aa, Artificial Sequence
  source: /note="Description of Artificial Sequence: Synthetic polypeptide"
QTVVTQEPSLTVSPGGTVTLTCRSSTGAVTTSNYANWVQQKPGQAPRGLIGGTNKRAPGTPARFSGSLLGGKAALTLSGVQPEDEAEYYCALWYSNLWVFGGGTKLTVLGQPKAAPSVTLFPPSSEELQANKATLVCLISDFYPGAVTVAWKADSSPVKAGVETTTPSKQSNNKYAASSYLSLTPEQWKSHRSYSCQVTHEGSTVEKTVAPTECS